European Patent Application EP 4 141 025 A1, published March 1, 2023. Title: A METHOD FOR PURIFYING OF BIOACTIVE PEPTIDE USING PROTEIN A AFFINITY CHROMATOGRAPHY. Applicant: ABL bio. The sequence listing filed with the application follows.

SEQUENCE LISTING (37 sequences)

SEQ ID NO: 1 - protein, 121 aa, Artificial Sequence
  H Variable region 1564
EVQLLESGGGLVQPGGSLRLSCAASGFTFSSYDMSWVRQAPGKCLEWVSAISYDNANTYYADSVKGRFTISRDNSKNTLYLQMNSLRAEDTAVYYCAKGVLTTLMNWFDYWGQGTLVTVSS

SEQ ID NO: 2 - protein, 110 aa, Artificial Sequence
  L Variable region 1564
QSVLTQPPSASGTPGQRVTISCTGSSSNIGSNDVSWYQQLPGTAPKLLIYANVNRPSGVPDRFSGSKSGTSASLAISGLRSEDEADYYCGAWDDSLNAYVFGCGTKLTVL

SEQ ID NO: 3 - protein, 121 aa, Artificial Sequence; identical to SEQ ID NO: 1
  H Variable region F06

SEQ ID NO: 4 - protein, 110 aa, Artificial Sequence
  L Variable region F06
QSVLTQPPSASGTPGQRVTISCTGSSSNIGSNDVSWYQQLPGTAPKLLIYANVNRPSGVPDRFSGSKSGTSASLAISGLRSEDEADYYCGTWAGSLNAYVFGCGTKLTVL

SEQ ID NO: 5 - protein, 121 aa, Artificial Sequence
  H Variable region VH5
EVQLLESGGGLVQPGGSLRLSCAASGFTFSSYDMSWVRQAPGKCLEWVSAISGDNASTYYADSVKGRFTISRDNSKNTLYLQMNSLRAEDTAVYYCAKGVLTTLMNWFDSWGQGTLVTVSS

SEQ ID NO: 6 - protein, 110 aa, Artificial Sequence; identical to SEQ ID NO: 2
  L Variable region VH5

SEQ ID NO: 7 - protein, 121 aa, Artificial Sequence
  H Variable region VH16
EVQLLESGGGLVQPGGSLRLSCAASGFTFSSYDMSWVRQAPGKCLEWVSAISGSNANTYYADSVKGRFTISRDNSKNTLYLQMNSLRAEDTAVYYCAKGVLTTLMNWFDYWGQGTLVTVSS

SEQ ID NO: 8 - protein, 110 aa, Artificial Sequence; identical to SEQ ID NO: 2
  L Variable region VH16

SEQ ID NO: 9 - protein, 121 aa, Artificial Sequence
  H Variable region VH9
EVQLLESGGGLVQPGGSLRLSCAASGFTFSSYDMSWVRQAPGKCLEWVSAISGDNGSTYYADSVKGRFTISRDNSKNTLYLQMNSLRAEDTAVYYCAKGVLTTLMNWFDSWGQGTLVTVSS

SEQ ID NO: 10 - protein, 110 aa, Artificial Sequence
  L Variable region VH9
QSVLTQPPSASGTPGQRVTISCTGSSSNIGSNDVSWYQQLPGTAPKLLIYANSNRPSGVSDRFSGSKSGTSASLAISGLRSEDEADYYCGAWDDSLNGYVFGCGTKLTVL

SEQ ID NO: 11 - protein, 251 aa, Artificial Sequence
  scFv 3_4
QSVLTQPPSASGTPGQRVTISCTGSSSNIGSNDVSWYQQLPGTAPKLLIYANVNRPSGVPDRFSGSKSGTSASLAISGLRSEDEADYYCGTWAGSLNAYVFGCGTKLTVLGGGGSGGGGSGGGGSGGGGSEVQLLESGGGLVQPGGSLRLSCAASGFTFSSYDMSWVRQAPGKCLEWVSAISYDNANTYYADSVKGRFTISRDNSKNTLYLQMNSLRAEDTAVYYCAKGVLTTLMNWFDYWGQGTLVTVSS

SEQ ID NO: 12 - protein, 716 aa, Artificial Sequence
  hu11F11(ver.2)(M428L)-F06(de2)(StoP)
EVQLVESGGGLVQPGGSLRLSCATSGFTFSDFYMEWVRQPPGKRLEWIAASRNKANDYTTEYSASVKGRFTVSRDDSKSSLYLQMNSLRAEDTAIYYCARDAHGKPFAYWGQGTTVTVSSASTKGPSVFPLAPSSKSTSGGTAALGCLVKDYFPEPVTVSWNSGALTSGVHTFPAVLQSSGLYSLSSVVTVPSSSLGTQTYICNVNHKPSNTKVDKKVEPKSCDKTHTCPPCPAPELLGGPSVFLFPPKPKDTLMISRTPEVTCVVVDVSHEDPEVKFNWYVDGVEVHNAKTKPREEQYNSTYRVVSVLTVLHQDWLNGKEYKCKVSNKALPAPIEKTISKAKGQPREPQVYTLPPSRDELTKNQVSLSCAVKGFYPSDIAVEWESNGQPENNYKTTPPVLDSDGSFFLVSKLTVDKSRWQQGNVFSCSVLHEALHNHYTQKSLSLSPGKGGGGSGGGGSGGGGSQSVLTQPPSASGTPGQRVTISCTGSSSNIGSNDVSWYQQLPGTAPKLLIYANVNRPSGVPDRFSGSKSGTSASLAISGLRSEDEADYYCGTWAGSLNAYVFGCGTKLTVLGGGGSGGGGSGGGGSGGGGSEVQLLESGGGLVQPGGSLRLSCAASGFTFSSYDMSWVRQAPGKCLEWVSAISYDNANTYYADSVKGRFTISRDNSKNTLYLQMNSLRAEDTAVYYCAKGVLTTLMNWFDYWGQGTLVTVSS

SEQ ID NO: 13 - protein, 450 aa, Artificial Sequence
  hu11F11(ver.2)(M428L)
EVQLVESGGGLVQPGGSLRLSCATSGFTFSDFYMEWVRQPPGKRLEWIAASRNKANDYTTEYSASVKGRFTVSRDDSKSSLYLQMNSLRAEDTAIYYCARDAHGKPFAYWGQGTTVTVSSASTKGPSVFPLAPSSKSTSGGTAALGCLVKDYFPEPVTVSWNSGALTSGVHTFPAVLQSSGLYSLSSVVTVPSSSLGTQTYICNVNHKPSNTKVDKKVEPKSCDKTHTCPPCPAPELLGGPSVFLFPPKPKDTLMISRTPEVTCVVVDVSHEDPEVKFNWYVDGVEVHNAKTKPREEQYNSTYRVVSVLTVLHQDWLNGKEYKCKVSNKALPAPIEKTISKAKGQPREPQVYTLPPSRDELTKNQVSLWCLVKGFYPSDIAVEWESNGQPENNYKTTPPVLDSDGSFFLYSKLTVDKSRWQQGNVFSCSVLHEALHNHYTQKSLSLSPGK

SEQ ID NO: 14 - protein, 15 aa, Artificial Sequence
  (G4S)3
GGGGSGGGGSGGGGS

SEQ ID NO: 15 - protein, 110 aa, Artificial Sequence; identical to SEQ ID NO: 4
  F06(de2)(StoP) VL

SEQ ID NO: 16 - protein, 20 aa, Artificial Sequence
  (G4S)4
GGGGSGGGGSGGGGSGGGGS

SEQ ID NO: 17 - protein, 121 aa, Artificial Sequence; identical to SEQ ID NO: 1
  F06(de2)(StoP) VH

SEQ ID NO: 18 - protein, 115 aa, Artificial Sequence
  ch1E4 VH
QVQLQQSGAELVRPGTSVKVSCKASGYAFTNYLIEWVKQRPGQGLEWIGVINPGSGGTNYNEKFKGKATLTADKSSSTAYMQLSSLTSDDSAVYFCASGNYDTYWGQGTLVTVSA

SEQ ID NO: 19 - protein, 112 aa, Artificial Sequence
  ch1E4 VL
DVVMTQTPLSLPVSLGDQASISCRSSQSLVHSNGNTYLHWYLQKPGQSPKLLIYKVSNRFSGVPDRFSGSGSGTDFTLKISRVEAEDLGVYFCSQSTHVPRTFGGGTKLEIK

SEQ ID NO: 20 - DNA, 2148 bp, Artificial Sequence
  hu11F11 F06 monovalent  conatant vector 1
gaggtgcagctcgtagagtcaggcgggggactcgtccaacccggtggttctcttagattgtcatgtgccacaagcggttttaccttttccgatttttacatggagtgggttcgtcagccaccagggaagcgacttgagtggatcgcagcatcccgtaataaggccaatgactatactaccgagtattccgcttcagtaaagggcagattcaccgtcagtagggatgacagcaagagcagcctctatctccagatgaatagtctgagggctgaagataccgccatttactactgtgcacgggatgctcatgggaagcccttcgcttactggggccaaggcaccactgtaaccgtatcctctgcctccaccaagggcccctccgtgttccccctggccccctcctccaagtccacctccggcggcaccgccgccctgggctgcctggtgaaggactacttccccgagcccgtgaccgtgtcctggaactccggcgccctgacctccggcgtgcacaccttccccgccgtgctgcagtcctccggcctgtactccctgtcctccgtcgtgaccgtgccctcctcctccctgggcacccagacctacatctgcaacgtgaaccacaagccctccaacaccaaggtggacaagaaggtggagcccaagtcctgcgacaagacccacacctgccctccctgccccgcccccgagctgctgggcggcccctccgtgttcctgttccctcctaagcccaaggacaccctgatgatctcccggacccccgaggtgacttgcgtggtggtggacgtgtcccacgaggaccccgaggtgaagttcaactggtacgtggacggcgtggaggtgcacaacgccaagaccaagccccgggaggagcagtacaactccacctaccgggtggtgtccgtgctgaccgtgctgcaccaggactggctgaacggcaaggagtacaagtgcaaggtgtccaacaaggccctgcccgcccccatcgagaagaccatctccaaggccaagggccagccccgggagccccaggtgtacaccctgcccccctcccgggatgaacttactaagaaccaggtctctctgtcatgcgccgtcaaaggtttttatccatccgacattgccgtcgagtgggagtcaaatggtcagccagagaataactacaagacaactccacccgtgctcgactccgacggcagcttctttttggtgtccaagttgaccgttgacaagtctcgttggcaacagggtaacgtattttcctgtagtgtccttcacgaggccctgcataaccactatactcaaaaatctctgtccctgagccctggaaaaggtggcggaggatctggcggtggtggttctggcggaggcggatctcagtctgttctgacccagcctccttctgcttctggcacccctggccagagagtgaccatctcttgtaccggctcctcctccaacatcggctccaacgacgtgtcctggtatcagcagctgcctggcacagcccctaaactgctgatctacgccaacgtaaaccggccttctggcgtgcctgacagattctccggctccaagtctggcacctctgcctccctggctatctccggcctgagatctgaggacgaggccgattactactgcggcacctgggccggatctctgaacgcctatgtgttcggctgcggcacaaagctgacagtgttgggaggcggaggaagtggtggcggcggttcaggcggcggtggcagcggaggtggtggatctgaagttcagctgctggaatctggcggcggattggttcagcctggtggctctctgagactgtcttgtgccgcctctggcttcaccttctccagctacgatatgtcctgggtccgacaggcccctggcaagtgtttggagtgggtgtccgccatctcctacgacaacgccaacacctactacgccgactccgtgaagggccggttcaccatctctcgggacaacagcaagaacaccctgtacctgcagatgaactccctgagagccgaggacaccgccgtgtactattgtgctaagggcgtgctgaccaccctgatgaattggttcgattactggggccagggcaccctggtcaccgtgtcatct

SEQ ID NO: 21 - DNA, 1350 bp, Artificial Sequence
  hu11F11 F06 monovalent  conatant vector 2
gaggtgcagctcgtagagtcaggcgggggactcgtccaacccggtggttctcttagattgtcatgtgccacaagcggttttaccttttccgatttttacatggagtgggttcgtcagccaccagggaagcgacttgagtggatcgcagcatcccgtaataaggccaatgactatactaccgagtattccgcttcagtaaagggcagattcaccgtcagtagggatgacagcaagagcagcctctatctccagatgaatagtctgagggctgaagataccgccatttactactgtgcacgggatgctcatgggaagcccttcgcttactggggccaaggcaccactgtaaccgtatcctctgcctccaccaagggcccctccgtgttccccctggccccctcctccaagtccacctccggcggcaccgccgccctgggctgcctggtgaaggactacttccccgagcccgtgaccgtgtcctggaactccggcgccctgacctccggcgtgcacaccttccccgccgtgctgcagtcctccggcctgtactccctgtcctccgtcgtgaccgtgccctcctcctccctgggcacccagacctacatctgcaacgtgaaccacaagccctccaacaccaaggtggacaagaaggtggagcccaagtcctgcgacaagacccacacctgccctccctgccccgcccccgagctgctgggcggcccctccgtgttcctgttccctcctaagcccaaggacaccctgatgatctcccggacccccgaggtgacttgcgtggtggtggacgtgtcccacgaggaccccgaggtgaagttcaactggtacgtggacggcgtggaggtgcacaacgccaagaccaagccccgggaggagcagtacaactccacctaccgggtggtgtccgtgctgaccgtgctgcaccaggactggctgaacggcaaggagtacaagtgcaaggtgtccaacaaggccctgcccgcccccatcgagaagaccatctccaaggccaagggccagccccgggagccccaggtgtacaccctgcccccctcccgtgatgaactcactaagaatcaagtcagtctctggtgtttggtcaaaggcttctatccatctgatattgctgttgaatgggagagtaacgggcaacctgaaaataattacaagactacacctcccgtgcttgattccgacggttccttctttctgtattccaagctgacagttgataagagtcgctggcagcaggggaacgtatttagttgttctgtacttcacgaagctctccataaccattacactcaaaagtccctgtccctgtcccccggcaag

SEQ ID NO: 22 - DNA, 660 bp, Artificial Sequence
  hu11F11 F06 monovalent  variable vector
gatatcgtgatgacccagtctccttcctctctggctgtgtccctgggcgagcgcgtcaccatgtcctgcaagtcctctcagtccctgctgtactcctccaaccagaagaactacctggcctggtatcagcagaagcccggccagtctccaaagctgctgatctactgggcctccaccagagaatctggcgtgccagatagattcaccggctctggctctggcaccgacttcaccctgacaatctcttccgtgaaggccgaggacgtggccgtgtactactgccagcagtactacagctacccctggacctttggcggaggcaccaagctggaaatcaagcggaccgtggccgctccctccgtgttcatcttcccaccctccgacgagcagctgaagtccggcaccgcttccgtcgtgtgcctgctgaacaacttctacccccgcgaggccaaggtgcagtggaaggtggacaacgccctgcagtccggcaactcccaggaatccgtcaccgagcaggactccaaggacagcacctacagcctgtcctccaccctgaccctgtccaaggccgactacgagaagcacaaggtgtacgcctgcgaagtgacccaccagggcctgtccagccccgtgaccaagtccttcaaccggggcgagtgc

SEQ ID NO: 23 - protein, 8 aa, Artificial Sequence
  human VH3 domain sequence
LYLQMNSL

SEQ ID NO: 24 - protein, 8 aa, Artificial Sequence
  human VH3 domain sequence
NYLQMNSL

SEQ ID NO: 25 - protein, 8 aa, Artificial Sequence
  human VH3 domain sequence
LHLQMNSL

SEQ ID NO: 26 - protein, 8 aa, Artificial Sequence
  human VH3 domain sequence
LYLQMDSL

SEQ ID NO: 27 - protein, 8 aa, Artificial Sequence
  human VH3 domain sequence
AYLQMNSL

SEQ ID NO: 28 - protein, 8 aa, Artificial Sequence
  human VH3 domain sequence
TYLQMNSL

SEQ ID NO: 29 - protein, 8 aa, Artificial Sequence
  human VH3 domain sequence
MYLQMSNL

SEQ ID NO: 30 - protein, 8 aa, Artificial Sequence
  human VH3 domain sequence
LYLQMSSL

SEQ ID NO: 31 - protein, 8 aa, Artificial Sequence
  human VH3 domain sequence
MYLQMNNL

SEQ ID NO: 32 - protein, 8 aa, Artificial Sequence
  human VH3 domain sequence
LYLQVNSL

SEQ ID NO: 33 - protein, 8 aa, Artificial Sequence
  human VH3 domain sequence
LYLQTNSL

SEQ ID NO: 34 - protein, 8 aa, Artificial Sequence
  human VH3 domain sequence
LFLQMNSL

SEQ ID NO: 35 - protein, 8 aa, Artificial Sequence
  human VH3 domain sequence
LYVQMSSL

SEQ ID NO: 36 - protein, 8 aa, Artificial Sequence
  human VH3 domain sequence
LYLQMGSL

SEQ ID NO: 37 - protein, 8 aa, Artificial Sequence
  human VH3 domain sequence
MYLQMNSL